European Patent Application EP 4 692 118 A1, published February 11, 2026. Title: ADAM9-TARGETING HUMANIZED ANTIBODY AND ANTIBODY-DRUG CONJUGATE COMPRISING SAME AND USE THEREOF. Applicant: DUALITY BIOLOGICS (SUZHOU) CO., LTD. The sequence listing filed with the application follows.

SEQUENCE LISTING (53 sequences)

SEQ ID NO: 1 - protein, 5 aa, synthetic construct
LYWMN

SEQ ID NO: 2 - protein, 5 aa, synthetic construct
LYWMD

SEQ ID NO: 3 - protein, 5 aa, synthetic construct
LYWMH

SEQ ID NO: 4 - protein, 5 aa, synthetic construct
LYWME

SEQ ID NO: 5 - protein, 17 aa, synthetic construct
RIIPIFGHTDYNEKFKD

SEQ ID NO: 6 - protein, 17 aa, synthetic construct
DIIPIFGHTKYEEKFRD

SEQ ID NO: 7 - protein, 17 aa, synthetic construct
RIIPIFGHTKYNEKFKD

SEQ ID NO: 8 - protein, 17 aa, synthetic construct
RIIPIFGHTKYNEKFKN

SEQ ID NO: 9 - protein, 17 aa, synthetic construct
DIIPIFGHTKYNEKFKD

SEQ ID NO: 10 - protein, 17 aa, synthetic construct
DIIPIFGHTKYNEKFRD

SEQ ID NO: 11 - protein, 14 aa, synthetic construct
GGYYYYPREGFLDY

SEQ ID NO: 12 - protein, 15 aa, synthetic construct
RSSQSVDYSGDSYMN

SEQ ID NO: 13 - protein, 15 aa, synthetic construct
RSDQSVDYSGDSYMN

SEQ ID NO: 14 - protein, 15 aa, synthetic construct
RASQSVDYSGDSYMN

SEQ ID NO: 15 - protein, 15 aa, synthetic construct
RASQSVDYSGDSYMD

SEQ ID NO: 16 - protein, 7 aa, synthetic construct
AASDRES

SEQ ID NO: 17 - protein, 7 aa, synthetic construct
AASDLES

SEQ ID NO: 18 - protein, 7 aa, synthetic construct
AASDRDS

SEQ ID NO: 19 - protein, 9 aa, synthetic construct
QQSREDPFT

SEQ ID NO: 20 - protein, 5 aa, synthetic construct
  VARIANT 5: note = X is X1, which is N, D, H or E.
LYWMX

SEQ ID NO: 21 - protein, 17 aa, synthetic construct
  VARIANT 1: note = X is X2, which is D or R.
  VARIANT 10: note = X is X3, which is K or D.
  VARIANT 12: note = X is X4, which is N or E.
  VARIANT 16: note = X is X5, which is R or K.
  VARIANT 17: note = X is X6, which is D or N.
XIIPIFGHTXYXEKFXX

SEQ ID NO: 22 - protein, 123 aa, synthetic construct
QVQLQESGAEVKRPGSSVKVSCKASGFTFPLYWMNWVRQRPGQGLEWMGRIIPIFGHTDYNEKFKDRATITRDESSNTAYMELSRLRSEDSAVYYCARGGYYYYPREGFLDYWGQGTSVTVSS

SEQ ID NO: 23 - protein, 111 aa, synthetic construct
DIVMTQSPASLSVSPGERASISCRSSQSVDYSGDSYMNWYQQKPGQSPRLLIYAASDRESGVPDRFSGSGSGTDFTLKISRVEEEDAGTYYCQQSREDPFTFGQGTKVDIK

SEQ ID NO: 24 - protein, 123 aa, synthetic construct
EVQLQESGSEVRRPSESVKMSCKDSGFTFPLYWMDWVRQRQGKSLEWMGDIIPIFGHTKYEEKFRDRATMDRDESSDTAYMELRRLRSDDSAVYYCARGGYYYYPREGFLDYWGQGTSVTVSS

SEQ ID NO: 25 - protein, 111 aa, synthetic construct
DIVMTQSPDSLSVSPGERATINCRSSQSVDYSGDSYMNWYQQKPGQSPRLLIYAASDRESGVPDRFSGSGSGTDFTLKISRVEEEDAATYYCQQSREDPFTFGQGTRVEIK

SEQ ID NO: 26 - protein, 123 aa, synthetic construct
QVQLQESGAELKKPGASVKVSCKASGFTFPLYWMHWVRQRTGRGLEWMGRIIPIFGHTKYNEKFKDRATITRDESSNTAYMELSSLTSEDSAVYYCARGGYYYYPREGFLDYWGQGTSVTVSS

SEQ ID NO: 27 - protein, 111 aa, synthetic construct
DIVMTQSPDSLSASPGERATLSCRSSQSVDYSGDSYMNWYQQKPGQSPKLLLYAASDRESGVPDRFSGSGSGTDFTLNINRVEEEDEATYYCQQSREDPFTFGQGTRVEIK

SEQ ID NO: 28 - protein, 123 aa, synthetic construct
QVQLQESGAEVKRPGSSVKVSCKASGFTFPLYWMNWVRQRPGRGLEWMGRIIPIFGHTKYNEKFKDRATMTRDKSSSTAYMELSSLTSDDSAVYYCARGGYYYYPREGFLDYWGQGTSVTVSS

SEQ ID NO: 29 - protein, 111 aa, synthetic construct
DIVMTQSPSSLSVSPGERATINCRSSQSVDYSGDSYMNWYQQKPGQAPRLLIYAASDLESGVPDRFSGSGSGTDFTLNINGVEEEDAATYYCQQSREDPFTFGQGTKVEIK

SEQ ID NO: 30 - protein, 111 aa, synthetic construct
DIVMTQSPDSLSVSPGERATINCRSSQSVDYSGDSYMNWYQQKPGQSPKLLIYAASDRESGVPDRFSGSGSGTDFTLNISRVEEEDAATYYCQQSREDPFTFGQGTRVEIK

SEQ ID NO: 31 - protein, 123 aa, synthetic construct
QVQLQQPGTEVVKPGASVKLSCKASGFTFPLYWMHWVRQRPGRGLEWIGRIIPIFGHTKYNEKFKNKATLTADESSSTAYMELRSLTSDDSAVYYCARGGYYYYPREGFLDYWGQGTSVTVSS

SEQ ID NO: 32 - protein, 111 aa, synthetic construct
DIVMTQSPASLSVSPGERASISCRSSQSVDYSGDSYMNWYQQKPGQSPRLLIYAASDRDSGVPDRFSGSGSGTDFTLKISRVEEEDAATYYCQQSREDPFTFGQGTRVEVK

SEQ ID NO: 33 - protein, 111 aa, synthetic construct
DIVMTQSPASLSVSPGERASINCRSDQSVDYSGDSYMNWYQQKPGKSPRLLIYAASDRESGVPDRFSGSGSGTDFTLNINSVEEEDAGTYYCQQSREDPFTFGQGTRVDIK

SEQ ID NO: 34 - protein, 123 aa, synthetic construct
QVQLQQPGAELKKPGASVKVSCKTSGFTFPLYWMHWVKQRPGRGLEWMGRIIPIFGHTKYNEKFKDKATLTRDESSSTAYMELSSLTSEDSAVYYCARGGYYYYPREGFLDYWGQGTSVTVSS

SEQ ID NO: 35 - protein, 111 aa, synthetic construct
DIVMTQSPSSLSASPGERASISCRSSQSVDYSGDSYMNWYQQRPGQSPRLLIYAASDRESGVPDRFSGSGSGTDFTLKISDVEEEDAATYYCQQSREDPFTFGQGTRVEIK

SEQ ID NO: 36 - protein, 123 aa, synthetic construct
QVQLQQSGTEVKRPGSSVKMSCKDSGFTFPLYWMDWVKQRHGRRLEWMGDIIPIFGHTKYNEKFKDRATMTTDESSSTAYMELRSLRSDDSAVYYCARGGYYYYPREGFLDYWGQGTSVTVSS

SEQ ID NO: 37 - protein, 123 aa, synthetic construct
QVQLQESGAELKRPGSSVKVSCKASGFTFPLYWMNWVRQRPGRGLEWMGRIIPIFGHTKYNEKFKDRATLTADESSSTAYMELSSLRSDDSAVYYCARGGYYYYPREGFLDYWGQGTSVTVSS

SEQ ID NO: 38 - protein, 111 aa, synthetic construct
DIVMTQSPASLSVSPGERASISCRSSQSVDYSGDSYMNWYQQKPGQSPRLLIYAASDRESGVPARFSGSKSGTDFTLKINRVEEEDAGTYYCQQSREDPFTFGQGTRVEIK

SEQ ID NO: 39 - protein, 123 aa, synthetic construct
QVQLQQSGAEVKRPGASVKMSCKASGFTFPLYWMNWVRQRPGRGLEWIGRIIPIFGHTKYNEKFKDRATITADESSDTAYMELSSLRSDDSAVYYCARGGYYYYPREGFLDYWGQGTSVTVSS

SEQ ID NO: 40 - protein, 111 aa, synthetic construct
DIVMTQSPDSLSVSPGERATINCRSDQSVDYSGDSYMNWYQQRPGQAPRLLIYAASDRESGTPDRFSGSGSGTDFTLNISRVEEEDAATYYCQQSREDPFTFGQGTRVEIK

SEQ ID NO: 41 - protein, 111 aa, synthetic construct
DIVMTQSPASLSVSPGERATLSCRASQSVDYSGDSYMNWYQQKPGQAPRLLIYAASDRDSGVPDRFSGSGSGTDFTLKINRVEEEDAATYYCQQSREDPFTFGQGTRVEIK

SEQ ID NO: 42 - protein, 123 aa, synthetic construct
QVQLQQPGAELKKPGASVKVSCKASGFTFPLYWMNWVRQRPGRGLEWIGRIIPIFGHTKYNEKFKDRATMTADESSSTAYMELSSLTSEDSAVYYCARGGYYYYPREGFLDYWGQGTSVTVSS

SEQ ID NO: 43 - protein, 111 aa, synthetic construct
DIVMTQSPDSLSVSPGERATINCRSSQSVDYSGDSYMNWYQQKPGQSPRLLIYAASDRESGVPDRFSGSGSGTDFTLKISNVEEEDAATYYCQQSREDPFTFGQGTRVEIK

SEQ ID NO: 44 - protein, 123 aa, synthetic construct
QMQLQESGAEVKKPSRSVRMSCKGSGFTFPLYWMEWVRQRPGKGLEWMGDIIPIFGHTKYNEKFRDRATMTRDESSNTAYMELRSLRSDDSAVYYCARGGYYYYPREGFLDYWGQGTSVTVSS

SEQ ID NO: 45 - protein, 111 aa, synthetic construct
DIVMTQSPDSLSVSPGQRASINCRSSQSVDYSGDSYMNWYQQRPGQAPRLLIYAASDRESGVPDRFSGSGSGTDFTLRINRVEEEDAGTYYCQQSREDPFTFGQGTRVDIK

SEQ ID NO: 46 - protein, 111 aa, synthetic construct
DIVMTQSPDSLSASVGDRASISCRASQSVDYSGDSYMDWYQQKPGQSPRLLIYAASDRESGVPDRFSGSGSGTDFTLKINRVEEEDAATYYCQQSREDPFTFGQGTRVEIK

SEQ ID NO: 47 - protein, 123 aa, synthetic construct
QVQLQQSGAEVRRPGSSVKMSCKDSGFTFPLYWMNWVRQRPGRGLEWMGRIIPIFGHTKYNEKFKDRATMTADESSSTAYMELSSLRSDDSAVYYCARGGYYYYPREGFLDYWGQGTSVTVSS

SEQ ID NO: 48 - protein, 330 aa, synthetic construct [sequence omitted]

SEQ ID NO: 49 - protein, 107 aa, synthetic construct [sequence omitted]

SEQ ID NO: 50 - protein, 453 aa, synthetic construct
QVQLQQPGTEVVKPGASVKLSCKASGFTFPLYWMHWVRQRPGRGLEWIGRIIPIFGHTKYNEKFKNKATLTADESSSTAYMELRSLTSDDSAVYYCARGGYYYYPREGFLDYWGQGTSVTVSSASTKGPSVFPLAPSSKSTSGGTAALGCLVKDYFPEPVTVSWNSGALTSGVHTFPAVLQSSGLYSLSSVVTVPSSSLGTQTYICNVNHKPSNTKVDKKVEPKSCDKTHTCPPCPAPELLGGPSVFLFPPKPKDTLMISRTPEVTCVVVDVSHEDPEVKFNWYVDGVEVHNAKTKPREEQYNSTYRVVSVLTVLHQDWLNGKEYKCKVSNKALPAPIEKTISKAKGQPREPQVYTLPPSRDELTKNQVSLTCLVKGFYPSDIAVEWESNGQPENNYKTTPPVLDSDGSFFLYSKLTVDKSRWQQGNVFSCSVMHEALHNHYTQKSLSLSPGK

SEQ ID NO: 51 - protein, 218 aa, synthetic construct
DIVMTQSPASLSVSPGERASISCRSSQSVDYSGDSYMNWYQQKPGQSPRLLIYAASDRESGVPDRFSGSGSGTDFTLKISRVEEEDAGTYYCQQSREDPFTFGQGTKVDIKRTVAAPSVFIFPPSDEQLKSGTASVVCLLNNFYPREAKVQWKVDNALQSGNSQESVTEQDSKDSTYSLSSTLTLSKADYEKHKVYACEVTHQGLSSPVTKSFNRGEC

SEQ ID NO: 52 - protein, 453 aa, synthetic construct
QVQLQQPGAELKKPGASVKVSCKASGFTFPLYWMNWVRQRPGRGLEWIGRIIPIFGHTKYNEKFKDRATMTADESSSTAYMELSSLTSEDSAVYYCARGGYYYYPREGFLDYWGQGTSVTVSSASTKGPSVFPLAPSSKSTSGGTAALGCLVKDYFPEPVTVSWNSGALTSGVHTFPAVLQSSGLYSLSSVVTVPSSSLGTQTYICNVNHKPSNTKVDKKVEPKSCDKTHTCPPCPAPELLGGPSVFLFPPKPKDTLMISRTPEVTCVVVDVSHEDPEVKFNWYVDGVEVHNAKTKPREEQYNSTYRVVSVLTVLHQDWLNGKEYKCKVSNKALPAPIEKTISKAKGQPREPQVYTLPPSRDELTKNQVSLTCLVKGFYPSDIAVEWESNGQPENNYKTTPPVLDSDGSFFLYSKLTVDKSRWQQGNVFSCSVMHEALHNHYTQKSLSLSPGK

SEQ ID NO: 53 - protein, 218 aa, synthetic construct
DIVMTQSPDSLSVSPGERATINCRSSQSVDYSGDSYMNWYQQKPGQSPRLLIYAASDRESGVPDRFSGSGSGTDFTLKISNVEEEDAATYYCQQSREDPFTFGQGTRVEIKRTVAAPSVFIFPPSDEQLKSGTASVVCLLNNFYPREAKVQWKVDNALQSGNSQESVTEQDSKDSTYSLSSTLTLSKADYEKHKVYACEVTHQGLSSPVTKSFNRGEC